European Patent Application EP 4 545 094 A2, published April 30, 2025. Title: Rekombinanter Orf-Virus-Vektor. Applicant: Prime Vector Technologies GmbH. Application EP. The sequence listing filed with the application follows.

SEQUENCE LISTING (6 sequences)

SEQ ID NO: 1 - DNA, 16 bp, synthetic construct
  misc_feature 1..16: note = P1 Promotor
  source 1..16: mol_type = other DNA
aaaaattgaaaaatta

SEQ ID NO: 2 - DNA, 16 bp, synthetic construct
  misc_feature 1..16: note = P2 Promotor
  source 1..16: mol_type = other DNA
aaaaattgaaattcta

SEQ ID NO: 3 - DNA, 16 bp, synthetic construct
  misc_feature 1..16: note = Optimisierter "early" Promotor
  source 1..16: mol_type = other DNA
aaaaattgaaaaayta

SEQ ID NO: 4 - DNA, 15 bp, synthetic construct
  misc_feature 1..15: note = 7.5 kDa Promotor
  source 1..15: mol_type = other DNA
aaaagtagaaaatta

SEQ ID NO: 5 - DNA, 16 bp, synthetic construct
  misc_feature 1..16: note = VEGF Promotor
  source 1..16: mol_type = other DNA
caaaatgtaaattata

SEQ ID NO: 6 - DNA, 16 bp, synthetic construct
  misc_feature 1..16: note = Consensus "early" Promotor
  source 1..16: mol_type = other DNA
aaaaaatgaaaaaawa